European Patent Application EP 4 544 912 A2, published April 30, 2025. Title: USE OF A STRUCTURAL POLYPEPTIDE FOR PLANT COATING. Applicant: AMSilk GmbH. Application EP, filed August 7, 2019. The sequence listing filed with the application follows.

SEQUENCE LISTING (4 sequences)

SEQ ID NO: 1 - protein, 35 aa, synthetic construct
  REGION 1..35: note = synthetic
  DOMAIN 1..35: note = Module C (ADF-4)
GSSAAAAAAAASGPGGYGPENQGPSGPGGYGPGGP

SEQ ID NO: 2 - protein, 35 aa, synthetic construct
  REGION 1..35: note = synthetic
  DOMAIN 1..35: note = Module Cc
GSSAAAAAAAASGPGGYGPENQGPCGPGGYGPGGP

SEQ ID NO: 3 - protein, 124 aa, synthetic construct
  REGION 1..124: note = based on ADF-3
  DOMAIN 1..124: note = NR3 (ADF-3)
GAASAAVSVGGYGPQSSSAPVASAAASRLSSPAASSRVSSAVSSLVSSGPTNQAALSNTISSVVSQVSASNPGLSGCDVLVQALLEVVSALVSILGSSSIGQINYGASAQYTQMVGQSVAQALA

SEQ ID NO: 4 - protein, 109 aa, synthetic construct
  REGION 1..109: note = based on ADF-4
  DOMAIN 1..109: note = NR4 (ADF-4)
GAYGPSPSASASVAASRLSSPAASSRVSSAVSSLVSSGPTNGAAVSGALNSLVSQISASNPGLSGCDALVQALLELVSALVAILSSASIGQVNVSSVSQSTQMISQALS